European Patent Application EP 4 379 050 A1, published June 5, 2024. Title: SUCROSE SYNTHETASE AND USE THEREOF. Applicant: ABIOCHEM BIOTECHNOLOGY CO., LTD. The sequence listing filed with the application follows.

SEQUENCE LISTING (29 sequences)

SEQ ID NO: 1 - DNA, 2427 bp, Artificial Sequence
  source 1..2427: mol_type = other DNA
atggctaacgctgaacgtatgatcacccgcgtgcactctcagcgtgaacgtctgaacgaaaccctggtgagcgaacgtaacgaagttctggctctgctgtctcgtgttgaagctaaaggtaaaggcatcctgcaacagaaccagatcattgcggagttcgaagcgctgccggaacagactcgcaaaaaactggaaggtggcccgttcttcgatcttctgaaaagcacccaggaagcgatcgtcctgccgccgtgggtggcgctggcggttcgtccgcgccctggtgtgtgggaatacctgcgcgtgaaccttcacgcactggttgtggaagaactgcaaccggccgagtttctgcactttaaagaagaactggtggacggcgttaaaaacggcaactttaccctggaactggatttcgaaccgttcaacgcaagcatcccgcgtccgaccctgcataaatacatcggcaacggcgtggacttcctgaaccgtcacctgagcgcgaaactgttccatgacaaagaaagcctcctgccgctgctgaaatttctgcgtctgcacagccatcaaggtaaaaacctgatgctgtctgaaaaaatccagaacctgaacaccctccagcacaccctgcgtaaagctgaagaatatctggcggaactgaaatccgagactctgtatgaagaatttgaagcgaaattcgaagaaattggtctggaacgtggctggggtgataacgcggaacgcgtgctcgatatgatccgcctgctgctggacctgctggaggcaccggacccgtgcaccctggaaaccttcctcggccgcgtaccgatggtttttaatgtagttatcctgtccccgcacggctactttgcgcaggacaatgtactgggttacccggacaccggtggccaggtggtctacattctggatcaggttcgtgcgctggaaatcgaaatgctgcaacgtatcaaacagcagggtctgaacattaaaccgcgcatcctgattctgacccgcctgctgccggatgccgtaggcaccacctgcggcgaacgcctggaacgcgtgtatgactctgaatactgtgacatcctgcgcgttccgttccgcaccgaaaaagggatcgtgcgtaaatggatcagccgcttcgaagtttggccgtacctggaaacttacaccgaagatgcggcagttgaactgtctaaagaactgaacggtaaaccggacctgatcatcggcaactactctgacggcaacttggtggcgagcctgctggctcacaaactgggcgttacccagtgcaccattgcacacgcactggaaaaaaccaaatacccggattccgatatttattggaaaaaactggacgataaataccacttcagctgccagttcaccgcggacatcttcgctatgaaccacaccgacttcatcatcacctccacctttcaggaaattgcaggttctaaagaaaccgtgggccagtacgaatcccacactgcattcactttaccaggtctgtatcgcgttgttcacggcatcgatgttttcgatccgaaattcaacatcgttagcccaggcgccgatatgagcatctatttcccgtacactgaagaaaaacgtcgtctgaccaaatttcactctgaaattgaagaactgctgtatagcgacgttgaaaacaaagaacatctgtgtgtgctgaaagataagaaaaaaccaatcctgttcacgatggcccgcctggaccgtgtgaaaaacctgtctggcctggtggaatggtacggtaaaaacacccgcttacgtgaactggcgaacctggtggttgttggtggtgaccgccgtaaagaatctaaagataacgaagaaaaagcggagatgaaaaagatgtatgatctgattgaagaatataaactgaacggccagttccgctggatttctagccagatggaccgcgttcgtaacggtgaactgtaccgttacatctgcgacaccaaaggtgcgtttgttcagccggctctgtatgaggcattcggtctgaccgttgttgaagcgatgacctgcggcctcccgaccttcgcgacgtgcaaaggcggtccggcggaaatcatcgttcacggcaaatctggtttccacattgacccgtaccacggcgatcaggcggctgataccctggctgacttctttaccaaatgcaaagaagatccgtcccactgggacgaaatctctaaaggtggtctgcaacgtattgaagaaaaatatacctggcagatctatagccagcgtctgctgaccctgaccggtgtttacggcttctggaaacatgtaagcaacctggatcgcctggaagcgcgtcgctacctggaaatgttctatgcgctgaaatatcgcccgctggcacaagcggtgccgctggcgcaggatgactaa

SEQ ID NO: 2 - DNA, 2418 bp, Artificial Sequence
  source 1..2418: mol_type = other DNA
atggctgaacgtgtgctgacccgtgtgcactccctgcgcgaacgcgttgatgcgaccctggccgcacaccgtaacgaaatcctgctgtttctgtctcgcattgaatcccacggcaaaggcattctgaaaccgcacgaactgctggccgaatttgacgcgattcgtcaggatgacaaaaacaaactgaacgaacacgcgttcgaagaactgctgaaatccactcaggaagcgatcgtgctgccgccgtgggtagctctggcaattcgtctgcgtccaggcgtgtgggaatacattcgtgtgaacgttaacgccctggtggtcgaagaactgagcgttccggaatatttgcagtttaaagaagaactggttgacggtgcctccaacggcaacttcgtgctggaactggactttgaaccgttcaccgcgtctttcccgaaaccgaccctgaccaaatccatcggtaacggtgttgagttcctgaaccgccacctgtccgcaaaaatgttccacgacaaagaaagcatgacccctctgctggaatttctgcgcgcacatcactataaaggtaaaaccatgatgctgaacgatcgcatccagaactccaacaccctccagaacgttctgcgtaaagcggaagaatacctgatcatgttgccgccggaaaccccgtacttcgagttcgaacacaaattccaggagatcggcctggagaaaggctggggcgacaccgccgaacgtgttcttgaaatggtgtgtatgttgctggatctgctggaagcgccggatagctgcaccctcgaaaaattcctgggtcgcatcccgatggtgtttaacgtcgttatcctgtctccgcacggttactttgctcaggagaacgtcctgggctatccggataccggcggccaggttgtatatatcctggaccaggttccggcgctggaacgtgaaatgctgaaacgtatcaaagaacagggcctggatattatcccgcgcattctgattgttacccgtctgctgccggacgcggtgggcaccacctgcggtcagcgtatcgaaaaagtgtacggtgcggaacactctcacattctgcgcgtgccatttcgcaccgaaaaaggcattgtgcgcaaatggatctcacgcttcgaagtttggccttacatggaaactttcatcgaagatgtggcgaaagagatctccgcagaactccaggcgaaaccggatctgatcatcggtaactattccgaaggcaacctggccgctagcctgctggcgcataaactgggcgttactcagtgcactattgcgcacgcgctggaaaaaaccaaatatccggattctgacatctactggaaaaaatttgatgaaaaataccacttctcaagccagtttaccgctgacctgatcgcaatgaaccacactgacttcatcatcacctccaccttccaggaaatcgctggttcaaaagacaccgtcggccagtacgaatcccacatggcgttcaccatgccgggtctgtatcgcgttgttcacggtattaacgtgttcgacccgaaatttaatatcgtgtcgccgggcgccgatattaacctgtacttcagctacagcgaaaccgaaaaacgcctgactgcgtttcacccggaaatcgacgaactgctgtattccgacgttgaaaacgatgaacacctgtgtgtgctgaaagatcgtaccaaaccgatcctgttcactatggcccgcctggatcgtgttaaaaacctgaccggtctggttgaatggtacgcgaaaaacccgcgtctgcgcggcctggtgaacctggttgtggtaggtggtgatcgccgtaaagaatctaaagatctggaagaacaggcggaaatgaagaaaatgtatgaactgatcgaaacccataacctgaacggccagtttcgttggatctctagccagatgaaccgcgttcgtaacggtgaactgtatcgttacatcgctgacaccaagggcgcgttcgttcagccggcattctacgaagcattcggcctgaccgttgtggaagctatgacctgcggtctgccgacttttgcgactaatcatggcggtccggccgagattatcgtacatggtaaatctggcttccacattgatccgtaccacggcgaacaggccgctgatctgctggctgatttctttgaaaaatgcaaaaaagacccgtcccattgggaaaccatttctatgggcggcctcaaacgtatcgaagaaaaatacacctggcagatctactctgaaagcctgctgaccctggcggctgtgtacggtttctggaaacatgtgtctaaactggatcgtctggaaatccgtcgctacctggaaatgttctacgcgctgaaataccgtaaaatggcggaagcggtgccgctggcggcggaataa

SEQ ID NO: 3 - DNA, 2460 bp, Artificial Sequence
  source 1..2460: mol_type = other DNA
atgcaccatcatcatcatcatggcggtagcggcatgacttgtgttctgttaaaagcagttgtagaaagcgacgaacgtgccgacctgcgccagttttcacgcattctgcaactgggcgaaaaacgctacctgctgcgcaacgacattctggatgcgtttgcagactattgccgcgatcaagaacgcccggtgccaccaccgagcgaaagccgtctgagcaaactggtcttctatacccaggaaattatcgtggataacgaatcactgtgttggatcgttcgtccacgtattgcacagcaggaagtgtgccgtttactggtcgaagacctgaccattgtgccgatgaccatcccggagctgctggatctgcgtgaccgcttggtgaaccattatcatccgaacgaaggcgacgtgtttgagattgatgtgcaaccgttttatgactatagcccaatcatccgtgatgcgaaaaacatcggtaagggcgtcgagttcctgaaccgctatcttagctcgaagctgttccaggacccgcgccaatggcaacagaacctgttcaacttcctgcgcattcatcgctacaatggctaccagctgctgattaacgagcgcattcgtagtccgcagcatctgagcgaacaggtcaaacaagcactggttgtgctgagcgatcgtccaccaactgaagcctatagcgagtttcgcttcgagctgcaaaacctgggttttgaaccaggttggggcaataccgttgcacgtgttcgtgacaccctggaaattctggaccagctgctggatagcccggaccatcaagttctggaagcgtttgtgagccgcatcccaatgctgttccgcattgcactgatttcgccgcatggttggttcggtcaggaaggtgttctgggtcgtccagatacgggtggtcaggttgtgtatatcctggaccaggtgaagagtctggagaaacagatgcgcgaagaccttgaactggccggtttaggcgttctggaagcacagccgaagatcatcgttctgacccgcctcattccaaatgcggaaggcaccctgtgtaaccaacgtctggaaaagatttacggcaccaatgatgcgtggattctgcgcgttccatttcgcgagttcaacccgaaagtcacgcagaattggattagccgctttgagatctggccgtacctggaaacctttgcgattgacgccgaacgtgaactgcgtgcagaatttggtcatgtaccggatctgatcatcggcaattatagcgacggtaatttggttgcgttcctgttagcgcgtcgcttaaaggtgacccagtgtaacatcgcacatgccctggaaaagagcaagtacctgtttagcaatctgtattggcaggatctggaagacaagtaccactttagcctgcaatttacagccgatctgattgcaatgaatgcagcgaatttcatcattagcagtacctaccaggagattgttggcactccggattccatcggtcaatacgagagctatcaatccttcaccatgccagacctgtaccatgtggttaatggcattgaactgttcagtccaaagtttaatgttgttccaccgggcgttaatgaacaggtgtattttccgtattatcattataccgaacgcctggaaggtgatcgccaacgcctggaagaactgctttttactctggaagatccgcagcagatttacggctacctggaagcacccgaaaaacgtccgttgttcagtatggctcgtctggatcgcatcaagaacctgaccggtttagccgaagcatttggccgtagcaaggcactgcaagaacgttgcaacctcattctggtagcgggcaaattacgcaccgcagatagcagcgaccgtgaagaaattgcggagatcgaaaaactgtaccagatcatccaccagtataacctgcatggcaagattcgttggcttggtattcgccttccgaaagccgatagcggcgaaatctaccgcattatcgcagatcgccagggcatttttgtgcaaccggcgttgtttgaagcgttcggcctgactattctggaggcgatgattagcggtctgccgacttttggcacccgcttcggtggtccgctggagatcatccaggatggtgtcaacggcttctacattaatccgactcatctggaagaaatggctgagacgattgtgcgcttcctggaagcatgtgaccgcgatccgcaggaatggcagcgcattagcaaggcgggcattgagcgtgtttatagcacctacacgtggaagatccattgcacccgcctgctgagcctggccaaaatctacggcttttggaattttagcagccaagaaaaccgcgaagatatgatgcgttacatggaagcactgttccatctgctgtataaaccgcgtgctcaggcactgctggccgaacatcttcagcgttaa

SEQ ID NO: 4 - DNA, 2382 bp, Artificial Sequence
  source 1..2382: mol_type = other DNA
atgtctgatgaactgcgtcgttacatcagccagaacagccactctgtttccggtctgctgcgtcacctgttcaacctccagcgcccgttcctgctgtacaccgacctccagaaagcgttcagccacttcgctgaagattacggtaacgatgcagacctggttgtgctccaggagttcttctctcgtctgcaagaggctgtactggctgaaccgtggatctgtctggcctggcgtccaggtccgggtcgctggaactacctgcgtctgcatcgtgaacagctgcacctggaaactctgactcctggcgactacctggcgtttaaagaaaaacaggttctgccggcgaacgaccaggaaccggtgctgaccgtggatttcgaagatttccgcgcggcgccgtaccgtctgcgtgatgaagctactattggtcagggtctggtatatatgaaccgtcgtctggcaggccagctgtttcgtgacatcaaagccggccgccaatctatcttggatttcctcgcggttcacaaactgaacggccagtccctgatggtgcgtgaccagccgccggattttgaaaccctgcgtcaaaccgttcagtacctgagcaccctgccgaaaaccaaaccgtggtctgaatttgctaccgaaatgagccgccgtggctttgctccgggctggggcgacattgctggccgcgttcgtgaaaccatgcgcctgctgatggatctgctggacgcgccgtctgcggaatctttagaagcgttcattgatcgcatcccgatgatcagccgcatcctgatcgtgagcatccacggctggttcgcccaggacaaagttctgggccgccctgatacgggcggccaggtggtgtacatcctggatcaggcccgtgctttagaacaggaaatgcgtcagcgtctggcgcatcagggcgtggatattgttccgcacattctgatcgctacgcgtctgattccggaagcagatggcacgacctgtgaccagcgcctggagtctgtgcacggtgcagacaacgtacgtatcctccgtgtcccgttccgccatccatctggtgaaatcctgccacactgggtgagccgttttaacgtttggccgtggctggaacactacgcggaggatcttgaacgcgaaaccttggcagaatttggtcgtcgcccagatctgattatcggtaattactcagacggtaatctggtagcctccatgctgtccgaacgcctgaacgtgacgcagtgcaatatcgcgcacgcgctggaaaaaagcaaatatctgtatagcgatctgtactggcgtgatcatgacgcgtcccaccacttcgcttgccagttcaccgcagatctgatcgcgatgaactctgcggacatcatcgttacctctacctatcaagaaatcgctggcaacgatcatgaagtaggccaatatgaaggtcatcagaactactccctgccgggcttataccgtgttgaaaacggcatcgatgtgttcgatactaaattcaacatcatcagtccgggtgcggatgcgcgttactacttcccgtactctgttagcgaggaacgtttacgtttcctgcacccggacattgatgcactgctgttcggtgaggagccggccgcagaccgtcgcggtgttctggaagatcgtaacaaaccgattattttctctatggcacgtatggatcacatcaaaaacctgagcggtctggctgaactcttcggcgctagcgaacgtctgcgtgaactggcaaacctggtgatcattggcggtcacgttaaccctcaggattctcaggacgaagaagaacgtggtcagatccaccgtatgcacggtattatggaccagtaccaactcgatggccagatgcgttggatcggttccctgctggacaaaaacgtggctggtgaactgtaccgcgttgttggtgatactcatggttgcttcgtgcagccggcgctgttcgaagcatttggtctgaccgtgattgaggcgatgtcgtctggtctgccggtattcgcaacccgttttggcggcccgctggaaatcatcgaggatggcatttcgggctttcacatcgatccgaacaaccagcaggaaaccgcgacccgcctggctgacttcctgggcgcggcggcggcggacattggcgtttgggaaaccatctccgatggcgccctggcacgcgttcgtgctcattatacctggggtcattacgccacccgtatgatgaccctggctcgtatcttcggcttctggcgtttcatgctgaaaaccgatcatcgcgcggcgcgtcgctatttgcagatgttccagcacctgcaatggcgcccgctggcgcacgcggttccgctgggtgaatcttaa

SEQ ID NO: 5 - DNA, 2385 bp, Artificial Sequence
  source 1..2385: mol_type = other DNA
atgaccaccatcgataccctggcgacctgcactcagcagaatcgtgatgcagtttatactctgctgcgtcgttacttcactgcgaaccgtaccctgctgttacagtctgatctgcgtgaaggcctgctgcaaaccgaacaggattgtggtcagtctgatatgctgcgtgcgttcgttttccgcctgcaagaaggcatcttctcttccccgtgggcgtacctggcactgcgtccagaaatcgctaaatgggagttcatgcgcatccaccaggaacacctgatcccggaaaaactgaccatttctgaatttctgaaattcaaagaaaccgtggtgaaaggcgaagctaccgaatccgtgttggaagttgacttcggcccattcaaccgcggcttcccgcgcctgaaagaaagccgtagcatcggtcagggcgttatctttctgaaccgtaaactgtctagtgaaatgttctcccgcattgaagcgggccacacctctctgttgcacttcctgggtgttcatgctatcgagggccagcagctgatgttttctaacaacagccacgacatccacgcggttcgtaaccagctgcgtcaggcgctggaaatgctggaaaccctggatggcaccacgccgtggattgaactcgcgccgaaaatgaaccaactgggcttcgcaccgggctggggccataatgctaaccgcgttgctgaaaccatgaacatgctgatggacattctggaagccccgtccccatccgcactggaagaatttctggcgtgcatcccgatgatcagccgtctgctgatcctttccccacacggctacttcggccaggacaacgttctgggtctgccagacaccggtggtcaggtggtgtatatcctggatcaggttcgtgccctggaaaaagaaatgcatgatcgcctccagcttcagggtgtacaggttgaaccgaaaatcctgatcgtgacccgtctgatcccggacgcaggtgatactacctgtaaccagcgtcttgaaaaagtgtccggttgcaccaacacctggatcttgcgtgtgccgttccgcaaacacaacggtgaaatcataccgcactggatcagccgcttcgagatttggccgcacctggaaatttttgcaggcgacgtcgaacgtgaagcactggcggagctgggcggccatccggatctgatcatcggtaactactccgatggcaacctggttgccactctgctgagccgtcgtctgggtgttacccagtgcaacattgctcacgcgctggaaaaaaccaaatacctgcactctgacatctactggcaggaaaatgaagataaatatcacttctcctgccagtacaccgccgatctgctggcgatgaactctgcggactttattgtgaccagcacctaccaggaaatcgctggtactcgtgaagcagaaggtcagtacgaatcctaccaggctttctcgatgccggacctgtaccgtgttattcatggcatcgacctgttcgatccgaaattcaatattgtttctcctggcgccaacgcagatatttacttcccgtacagcgatccgaaccgccgcctgcactcactgatcccggagatcgaaagcctgatttttgatgacgctactaatctgccggctcgtggttacttgcaggacccggacaaaccgctgatctttactatggcacgtctggatcgtattaaaaacatcaccggcttagtagaactgtatgccgctagcccgcgcctgcgctccctggcgaacctggtaattgttggcggtaaaatcgatccgcagcacagctctgaccacgaagaacaggaacagattcatcgtatgcaccaactgatggacgaacacgaactggaccagcaggttcgctggctgggtatgcgcctggacaaaaaccttgctggcgaactgtatcgttatattgcagataaacgtggcattttcgtgcagccggccctgttcgaagccttcggcctgaccatcatcgaagcgatggcgtccggcctgccgacctttgcaacccgttacggcggcccgttggaaatcattcagaacaaccgttctggtttccacatcgacccgaaccagggtgcggcaaccgcggacctgatcgcagatttcttcgagaaaaacctggaaaacccgcaggaatgggaacgtatttcccaaggtgcgctggatcgtgttgccagccgttacacctggaaactgtacgctgaacgtatgatgaccctgtcccgtatctatggcttttggaaattcgtaagcggtctggaacgtgaagaaaccgatcgctacctgaacatgttctaccacctccagttccgtccgctggctaaccgtctggcgcatgaaatctaa

SEQ ID NO: 6 - DNA, 2382 bp, Artificial Sequence
  source 1..2382: mol_type = other DNA
atgatcaaagacatctacaaaaccgcggaaaccttccataacgacttctacgacttcctgaaagccgttagcactcagccgaaaaaactgatgattaccggtgaactgattaacctgtatgttgcgagtggctatgataaaaactccggcctgtacgaatttattgaaaaaattcaagaaaccattagcctggaccatagcgtgattctggatgtgcgtatcaaaatcgcgtccattaaattttaccgcatttccctggaagagttcttgatcgaagaaatctcatctaaggaatttctcatttataaagaaaccgttgcgaaaccggataccctgaacaccaccctgaacctgaacttcaagccgttctacgacaaatccccggcggttcgtgatattaaatacatcggctctggtgttgaatacctgaaccgttttctgagtagccagatgttcactaacgaagaacgctggaagaaaaacctgttcgatttcatccgcctgcataacttcaacggtgagcagctgattctgaacgatcgcatcaaagacaccaaacatctgaacaaccagatcaacgcggcgctggcgaaactgggcaaccacccggccaataccccatacgaaaacattaaacacatcctccaggaactgggtttcgaaaaaggcctgggcaaagatgcgggtacgatcactcacaacctgaacctgttagaccagctgctgaactcaccggatcacaacgccctggcggagttcatctcctccatcccgatgatcctgaacatcgctatcatctccccgcacggcttcttcggtcaagaaggtgttctgggcctgccggataccggtggccaggtagtgtacatcctggatcaggtgaaagcactggagaaacagctcattgattccctgaagaaaagcggtctgaacctgctgccgaaaatcatcgtcctgacccgccttatcccgaacgctcgtggcaccacctgcaaccagcgtctggaaaaaatctatggcgcaaagaatagctggattctgcgcgttccgttccgcgaatacaataaacgcgtaactgatgaatggatctctcgtttcgaaatttggccgtacctggaagatttcgccgaggactcgtacaccgctctgctggctgaatttaaaaagcgcccggatctgatcatcggtaactattccgacggtaacctggtggcatacctgctcgcaaaaaagtttaaggttacccagtgcggcatcgcacacgcactcgaaaaatctaaatatctgtactccgcgctgtactggtacgatctggaaaaatattaccacttctctatgcagttcaccgcagatctcctggcgatcaatagcgccgacttcctgattaccagcagcttccaggaaatcgcgggcaccgaaaaatctatcggtcagtacgaatcttatatgcatttcacgatgccgggcctttatcgtgttgaaaacggcgttaacccgttccacgtgaaatttaacatcgttagcccaggcgttaacgaaaaaatctacttcccgtacccaaaaaccaaatggcgtctgaaagaaaccaaacgccgcattgaaaacctgttcttctccaactccgaggacccggatgttatcggctggctggacaacccggaaaaaactccgattttcactatgagccgtctggatcgtattaaaaacatctccttcctggttcgttgcttcggtgaaagcgaagaattgcagcagacctccaacctgattgtggtggctggtaaaattgatgaaaccatgaccgacgattatgaagaaaaagaacagatccgcctgatgcacgaacttattactaaatataaactgcataacaaaatccgttggatcggcaagctcctgccgaaagacgaatccggtgaagcgtaccgtattattgctgaacgccgtggcatcttcgtgcagccggcactgtttgagggctttggcctgaccgttctggaagctatgaccagtggcctgccggtttttgctactaaatacggtggcccgctggaaatcattcagaacggggtgaacggctttcacattgatccggtgaaccaagaagaaaccaccgaaaagattgttcgtttcctgtctgacagctatatcgatagctctgtttgggataaactgagcaaagcggcgatcaaacgtgtcaccgaaaaatatagctggaaactgtactctaaacgcctgctgagccttgcgaaactgtatggtttctggaaatacgcaaccaacctggaacatgaggacattaacgcttacctggacctgatctaccacaccatctacaaatctcgtgcgaaaatcctgctggaagaacacatgaaacgttaa

SEQ ID NO: 7 - DNA, 2361 bp, Artificial Sequence
  source 1..2361: mol_type = other DNA
atgaacctgagcaacaaagaactggaaggcctggatgaaatcatctctgaccatcgtgaagatttctgcccgttcctgggccgtatcgaagaagaggacaaacagttcttcctgtctagcgaaatgaaagaaatgtacgcgggtgataccgtgccggacttcatcgcatctctccaggaagcggttaaaatgccgggtcagatctacttcgcgacccgcgcgagcatcggtgaatgggcgtttgtgaccgtattcaccgacaccctggactacatggaagtttccccgaccgaataccaggaagcaaaagaaaaaaccgtcctgggcgaaaacgcagcgtggatgccgtctgttgacctgaaaccgtttaaccgtgatttcccgaaaccgagcagcgcggatttcatcggtaaaggtgtagagttcctgaaccgccatcagtctagtcgtatcttcatgaacccggaaaaaggcttaaaacagctcctggatttcctgcgcgttcacaaatatgatggccgccagctgatgctgaacaaccgtatcgatagcgtggataaactgaaaaaagcgctgaaaaaagcacaggccctgctgaaaaataaaagcgacgaaactgaatgggaagaagttgaaagcgatatggcccacctgggcttcgaaccgggctggggcaaaaaactgggttacgtgaaagaatttctggcgctgctgtctgacattctggcagcgccggaacctgttgttctggaaaaattcctggatcgcattccgatgatcttcagcttagtggtactgagcccgcacggcttcttcggccaggccggtgtttttggtaaaccggataccggtggccaggttgtgtatatcctggatcaggttaaagcgctggaacacgaactgaaatcacgtctggacgaaaaaggcctggatattaccccgaaaatcctggtggtgacgcgtctgatcccggaggcggaaggcaccaactgcgatatggaagaagaacttatccgtggcaccgataactgccacatcgtccgtgtgccgttccgtgatgaatccggcgaagtagttcgtcagtggatctctcgtttccgtatctggccgtacctggaacgttttagcaccgaagcccagaacatcatcctgtccaagctgcaaggtaacccggacctgatcatcggtaactattccgacggtaacctggtggcgagcctgattgcccagcgcctgggcgttacccagtgcaccattgcccacgcgctggaaaaaaccaaatacctgtactccgatctgtactggcaggacaacaacgacaaataccacttcgcttgccagtacaccgcggatttgatctccatgaactactctgatttcatcatcacttctacctatcaggaaatcgccggcaccaacgattccgtcggccagtacgaatcctatatgaactacaccctgccgggcctgtaccgtgtggtgaacggcattgacgtttttgatccgaaatttaacgttgttagtccgggtgcggcgccagacatcttcttctcttataaaagcaaagatcgtttcccggaacacatcgaagaaatcgagagcatcctgttcgaagataacctggaaggctctcgtggttccctggctgatccggataaaccactgatcttcacgatggctcgcctggacaaaattaaaaacctgaccggcctggttcgctggttcggtgaaaacgaagaactgcgcaaaaccgcaaacctgctggtaatcggcggcttcgttgatgaaagcctgagcagtgacgatgaagaacgcgaacagatccgtatcatgcacagcgtgatcgatgaactgggcctggatggcagcgtgcgctgggtgggtgcgcacctgggtaaacgcatgaccggtgagttctatcgctatgttgctgatcgtaaaggtgttttcgtgcagccggcgctgttcgaagcgtttggtctgaccatcatcgaagcgatgagcagcggcctgccggttttcgcgactgtgtacggcggcccgtctgaaattatcgaagatggcaaaagcggtttcaccctggacccgaacaaaggcgacgaatgcgcagaaaaactgctggagttcattcagaaatgccagtccgaccctggtcactggatcaaaatctccgataacgcgctgaaacgcgtggaggaacgttataactggccgctgtacgcgaaacgtctgatgaccttcgctcgcgtttacggcttctggaaattcgtgaccaacctggaacgtgaagaaaccgtgcgttatctggaaatgctgtacggcatggtgtaccgtcgtctggctgacccgaaagaatactaa

SEQ ID NO: 8 - DNA, 2425 bp, Artificial Sequence
  source 1..2425: mol_type = other DNA
catatgtccgaacgtgcgcgtagcgatgatctgattgaacagctgcgcggcttcctggatgcttgtccgtccgtgggtcatcgcgttctgcaccagattaaaaaactggaacgctccttccttcagcgttctgaactgtgcgacgcgtttgcagatgtttgcgcagccgaagatgttccagatggcctgcgccagagcccgctgggtaaagttattcgtctgacccaggaagccgctgttaacgatgcttgggtttacctggctgttcgtgtgcgtattgcgtcctggcgttacgttcgtatcgcgctggaaggtatggcggttgaagaagtgactgttcgtgatttcctgcgtttcaaagaatgtctggctttgggccagcacgattttgatgaatggctgctggaaattgatctgggtccgttctctcgtgaatttccgaaactgctggaagcccgttccattggccgtggtgttgaatttctgaacaaacatctgagcctgcaactgttcgacgaactgggtgaaggtggtgaacgcatcctgaacttcctgcgcatccactcttttcgcggccagaccctgatgctgaacgaacagattaaatccgtgtctgatctccgtcgtgcactgcgtcgtgcggatgaagtgttggccggtcacgagccgacggcgacctgggaagatgtggctgcaccgctgcgcgcactgggtttcgaagttggttggggtcgtgaagttgcgcgtatccgtgacaccatgagcctgctgcgtgatctgctggaagcaccagaccctcgtggcctggaaacctttctggctcgtctgccgatggtgttttctctggctatcatttctccgcacggttacttcggtcaggctaacgttctgggtcgtccggatactggtggtcaggtggtatacattctggaccaggttcgtgccctcgaaaccgagatgcgctctcgcctgttcgaacagggcctggacatcgaaccgcagattgttgtcctgacccgtctgatcccgcaggctgaaggcaccacctgcgatcagcgtctggaaccgatctctggcactcgcaacgcgcgcatcctgcgtgtcccgttccgtaacgccagcggtgaaatcgttacccactggatttctcgtttcgaggtgtggccttacctggaacgttacactctggatagcgaacgtgaactgctggctgaactgggtggccgtccggatctgatcgttggtaattatagcgacggtaacctggtggctaccctgctgtcccagcgcctgggcgtgacccagtgcaacatcgcacacgcgctggaaaaaaccaaataccgtcacgccgacctgttctggcaggaaaacgaagcgcagtatcattttagctgccagtttaccgcggatctgattgctatgaacgctgctgactttatcatcacgtctacctaccaggaaatcgctggtacgcgcgaatccgttggccagtatgagagccacaccgcgttcaccatgccgaaactgttccgtgtggtcaacggcattgacgtgtatgacccaaaattcaacatcgtgagtccgggcgccgacgcagctgcatacttcccgtataccgcggtggaacgtcgcctcccgcatctgcacactgaaatcgaacagctggttttcggcgtggatgaacgtgttgacgcgcgcggcgtgctgaccgaacgtgacaaaccgctgctgttcactatggctcgtttggaccgtatcaaaaacatcgttggtctggttgaatggttcggcgcgtgcgaagcgctgcgtaaagaagcgaatctgctggtcatctcaggtcacgtagacccggaacgctcatccgacactgaagaactggaacagatccgttgtatgcacgctctgttcaaccgttatgatctggatcgtcaggtgcgctggctgggtctgcgtctgccgaaagatctggcgggtgaattttaccgctatgttgcggacggtcgtggcgcgttcgttcagccggctctgtttgaagcattcggtctgaccgtgattgaagcgatggcgtctggcctgccgtgcttcgcaacctgcttcggcggcccgtctgaaatcattgaagatggtgtctctggcttccacatcgatccgaaccacggcgatgcggcagcggaacgtatcgcgcgctttttcgaacgtacccgtcaagatccggaatattggaaccgtatctctgaaggcgcgctgaaacgtgtggccgaacgctacacctggcagcattatgctgaacgtatgatgaccctgagccgtgtttacggcttctggcgtcatgttactgacctggaacgtcgtgaaacccagcgttacctgcaagctctgtattctctgcaattccgtcgtctggcgcaggcgatggcgtaagctt

SEQ ID NO: 9 - protein, 819 aa, Artificial Sequence
MHHHHHHGGSGMTCVLLKAVVESDERADLRQFSRILQLGEKRYLLRNDILDAFADYCRDQERPVPPPSESRLSKLVFYTQEIIVDNESLCWIVRPRIAQQEVCRLLVEDLTIVPMTIPELLDLRDRLVNHYHPNEGDVFEIDVQPFYDYSPIIRDAKNIGKGVEFLNRYLSSKLFQDPRQWQQNLFNFLRIHRYNGYQLLINERIRSPQHLSEQVKQALVVLSDRPPTEAYSEFRFELQNLGFEPGWGNTVARVRDTLEILDQLLDSPDHQVLEAFVSRIPMLFRIALISPHGWFGQEGVLGRPDTGGQVVYILDQVKSLEKQMREDLELAGLGVLEAQPKIIVLTRLIPNAEGTLCNQRLEKIYGTNDAWILRVPFREFNPKVTQNWISRFEIWPYLETFAIDAERELRAEFGHVPDLIIGNYSDGNLVAFLLARRLKVTQCNIAHALEKSKYLFSNLYWQDLEDKYHFSLQFTADLIAMNAANFIISSTYQEIVGTPDSIGQYESYQSFTMPDLYHVVNGIELFSPKFNVVPPGVNEQVYFPYYHYTERLEGDRQRLEELLFTLEDPQQIYGYLEAPEKRPLFSMARLDRIKNLTGLAEAFGRSKALQERCNLILVAGKLRTADSSDREEIAEIEKLYQIIHQYNLHGKIRWLGIRLPKADSGEIYRIIADRQGIFVQPALFEAFGLTILEAMISGLPTFGTRFGGPLEIIQDGVNGFYINPTHLEEMAETIVRFLEACDRDPQEWQRISKAGIERVYSTYTWKIHCTRLLSLAKIYGFWNFSSQENREDMMRYMEALFHLLYKPRAQALLAEHLQR

SEQ ID NO: 10 - protein, 794 aa, Artificial Sequence
MTTIDTLATCTQQNRDAVYTLLRRYFTANRTLLLQSDLREGLLQTEQDCGQSDMLRAFVFRLQEGIFSSPWAYLALRPEIAKWEFMRIHQEHLIPEKLTISEFLKFKETVVKGEATESVLEVDFGPFNRGFPRLKESRSIGQGVIFLNRKLSSEMFSRIEAGHTSLLHFLGVHAIEGQQLMFSNNSHDIHAVRNQLRQALEMLETLDGTTPWIELAPKMNQLGFAPGWGHNANRVAETMNMLMDILEAPSPSALEEFLACIPMISRLLILSPHGYFGQDNVLGLPDTGGQVVYILDQVRALEKEMHDRLQLQGVQVEPKILIVTRLIPDAGDTTCNQRLEKVSGCTNTWILRVPFRKHNGEIIPHWISRFEIWPHLEIFAGDVEREALAELGGHPDLIIGNYSDGNLVATLLSRRLGVTQCNIAHALEKTKYLHSDIYWQENEDKYHFSCQYTADLLAMNSADFIVTSTYQEIAGTREAEGQYESYQAFSMPDLYRVIHGIDLFDPKFNIVSPGANADIYFPYSDPNRRLHSLIPEIESLIFDDATNLPARGYLQDPDKPLIFTMARLDRIKNITGLVELYAASPRLRSLANLVIVGGKIDPQHSSDHEEQEQIHRMHQLMDEHELDQQVRWLGMRLDKNLAGELYRYIADKRGIFVQPALFEAFGLTIIEAMASGLPTFATRYGGPLEIIQNNRSGFHIDPNQGAATADLIADFFEKNLENPQEWERISQGALDRVASRYTWKLYAERMMTLSRIYGFWKFVSGLEREETDRYLNMFYHLQFRPLANRLAHEI

SEQ ID NO: 11 - protein, 805 aa, Artificial Sequence
MSERARSDDLIEQLRGFLDACPSVGHRVLHQIKKLERSFLQRSELCDAFADVCAAEDVPDGLRQSPLGKVIRLTQEAAVNDAWVYLAVRVRIASWRYVRIALEGMAVEEVTVRDFLRFKECLALGQHDFDEWLLEIDLGPFSREFPKLLEARSIGRGVEFLNKHLSLQLFDELGEGGERILNFLRIHSFRGQTLMLNEQIKSVSDLRRALRRADEVLAGHEPTATWEDVAAPLRALGFEVGWGREVARIRDTMSLLRDLLEAPDPRGLETFLARLPMVFSLAIISPHGYFGQANVLGRPDTGGQVVYILDQVRALETEMRSRLFEQGLDIEPQIVVLTRLIPQAEGTTCDQRLEPISGTRNARILRVPFRNASGEIVTHWISRFEVWPYLERYTLDSERELLAELGGRPDLIVGNYSDGNLVATLLSQRLGVTQCNIAHALEKTKYRHADLFWQENEAQYHFSCQFTADLIAMNAADFIITSTYQEIAGTRESVGQYESHTAFTMPKLFRVVNGIDVYDPKFNIVSPGADAAAYFPYTAVERRLPHLHTEIEQLVFGVDERVDARGVLTERDKPLLFTMARLDRIKNIVGLVEWFGACEALRKEANLLVISGHVDPERSSDTEELEQIRCMHALFNRYDLDRQVRWLGLRLPKDLAGEFYRYVADGRGAFVQPALFEAFGLTVIEAMASGLPCFATCFGGPSEIIEDGVSGFHIDPNHGDAAAERIARFFERTRQDPEYWNRISEGALKRVAERYTWQHYAERMMTLSRVYGFWRHVTDLERRETQRYLQALYSLQFRRLAQAMA

SEQ ID NO: 12 - DNA, 1350 bp, Artificial Sequence
  source 1..1350: mol_type = other DNA
atgcaccatcatcatgaaggcgtgagcgaccagaccctgagagtaacgatgtttccgtggcttgggctgggtcatgttaacccgtttttgcgtatcgctaaacaactggccgatcgtggtttcgttatctatttagttagtaccgctattaacctcgaaatgatcaaaaagagaatcccggagaaatacagtaatagcatccatctggttgagctgcgcctgccagaattaccggaactgccaccacattaccatactaccaacggtttaccaccgcatctgaacaaaaccctgcacaaggcactgaagatgagcgctcccaactttagcaagatccttcaaaatattaagccggacctggtcctttacgattttctggttccgtgggcagaaaaagtcgcgcttgaacagggcatcccggctgttccattgctaaccagtggtgcggcactgttcagctactttttcaacttcctgaagcgaccgggtgaagagtttccgtttgaggcaatccgcctgtcgaagcgagaacaggataagatgcgcgagatgtttggaacagagccgcctgaagaagattttttagcgccggcccaggccggtatcatgctgatgtgcacgagccgcgtaattgaggctaagtacctggactattgtaccgaactgaccaatgtaaaagttgttccggttggtccgccgtttcaggatccgctgaccgaagatattgacgaccccgaactgatggattggttagataccaaacccgaacatagtgttgtctatgtgtcgtttggcagcgaagcgttcctgagccgtgaagatatggaagaagtcgcgttcggcctggagctgagcggcgtgaactttatctgggttgcacgctttccgaaaggcgaagaacagcgtctggaagacgttctgccaaaaggcttcctggaacgcgttggtgatcgtggtcgcgttctggaccatctggtgccgcaggcccatattctgaaccatccgagcacgggtggcttcatctctcattgcggttggaacagcgtcatggaaagcattgatttcggcgttccgatcattgcgatgccgatgcagtgggatcagccgattaacgcgagactgcttgtggaattaggcgtggcagtggagatcccgcgtgatgaagatggccgggtccaccgcgccgaaattgcccgtgtcctgaaagatgtgatttcgggcccgactggtgagatactgcgcgcgaaagtacgcgacattagcgcacgcctgagagcgagacgcgaggaggaaatgaacgcagcggcggaagaactgatacagctgtgtcgcaaccgcaacgcctacaag

SEQ ID NO: 13 - DNA, 30 bp, Artificial Sequence
  source 1..30: mol_type = other DNA
aaaaaactggtacgctccttccttcagcgt

SEQ ID NO: 14 - DNA, 30 bp, Artificial Sequence
  source 1..30: mol_type = other DNA
aaggagcgtaccagttttttaatctggtgc

SEQ ID NO: 15 - DNA, 30 bp, Artificial Sequence
  source 1..30: mol_type = other DNA
ttcagcgtgaagaactgtgcgacgcgtttg

SEQ ID NO: 16 - DNA, 31 bp, Artificial Sequence
  source 1..31: mol_type = other DNA
gcacagttcttcacgctgaaggaaggagcgt

SEQ ID NO: 17 - DNA, 30 bp, Artificial Sequence
  source 1..30: mol_type = other DNA
ggtggtgaagccatcctgaacttcctgcgc

SEQ ID NO: 18 - DNA, 31 bp, Artificial Sequence
  source 1..31: mol_type = other DNA
gttcaggatggcttcaccaccttcacccagt

SEQ ID NO: 19 - DNA, 29 bp, Artificial Sequence
  source 1..29: mol_type = other DNA
gttacactcgggatagcgaacgtgaactg

SEQ ID NO: 20 - DNA, 31 bp, Artificial Sequence
  source 1..31: mol_type = other DNA
gttcgctatcccgagtgtaacgttccaggta

SEQ ID NO: 21 - DNA, 30 bp, Artificial Sequence
  source 1..30: mol_type = other DNA
accaaataccctcacgccgacctgttctgg

SEQ ID NO: 22 - DNA, 30 bp, Artificial Sequence
  source 1..30: mol_type = other DNA
gtcggcgtgagggtatttggttttttccag

SEQ ID NO: 23 - DNA, 31 bp, Artificial Sequence
  source 1..31: mol_type = other DNA
gttctggcagctaaacgaagcgcagtatcat

SEQ ID NO: 24 - DNA, 30 bp, Artificial Sequence
  source 1..30: mol_type = other DNA
gcttcgtttagctgccagaacaggtcggcg

SEQ ID NO: 25 - DNA, 30 bp, Artificial Sequence
  source 1..30: mol_type = other DNA
ctgccgaaacgtctggcgggtgaattttac

SEQ ID NO: 26 - DNA, 29 bp, Artificial Sequence
  source 1..29: mol_type = other DNA
ccgccagacgtttcggcagacgcagaccc

SEQ ID NO: 27 - DNA, 19 bp, Artificial Sequence
  source 1..19: mol_type = other DNA
gcccgacattatcgcgagc

SEQ ID NO: 28 - DNA, 19 bp, Artificial Sequence
  source 1..19: mol_type = other DNA
gggtataaatgggctcgcg

SEQ ID NO: 29 - DNA, 1371 bp, Artificial Sequence
  source 1..1371: mol_type = other DNA
atgccgaacactaacccaactaccgtgcgtcgtcgtcgtgttattatgtttccggttccgttcccgggccacttaaacccgatgctgcaactggcgaacgtgctgtaccgtagaggttttgaaatcaccattctgcacaccaacttcaacgccccgaaaaccagcctttatccgcacttccagtttcgttttatcttggacaacgatccgcaaccggagtggttacgcaacctgccgacgactggtccgggcgtgggtgcaagaatcccggtaattaacaaacacggcgcggatgaattccgtaaggagctggaaatctgcatgcgggatactccgagtgacgaggaagttgcttgcgtgattaccgatgcgctgtggtacttcgcgcaaccggtggcggacagcctgaatctgaaacgtctggttctgcagaccgggagcctgtttaacttccactgcctggtgtgtctgccgaaatttctggagttgggctacctggatccggaaactaaacatcgtccggatgaaccggtggtaggtttcccgatgctgaaggttaaagatatccgtcgcgcgtattcgcacattcaagaatcgaaaccaattctgatgaagatggttgaagaaacccgtgccagcagcggtgtgatttggaacagcgctaaagagctggaggaaagcgagctggaaaccattcagcgtgaaattccggcgccgagcttcctgcttccgctgccgaagcattatagggcttcgagcactagcctgctggatactgatccgagcaccgcccaatggctggaccagcagccgccgagcagcgtgctgtacgttggctttggcagccagagctcgctggaccccgcagatttcctggagattgcgcgtggtctggttgcgagcaaacaaagctttctgtggctggttcgtccgggcttcgtgaagggttatgagtggattgagctgctgccggatggttttctgggtgaaaaaggtcgtatcgtgaagtctgctccgcaacaagaagtgctggcgcacaaggcgattggtgcgttctggacccacggcggttggaacggcaccatggaggccgtgtgcgaaggcgtgccgatgatctttagcgatttcggtctggatcagccgctgaacgcgcgttacatgagcgaggttctgcatgtgggcgtttatctggagaacggcttcatccgtggtgagatcattaatgcggttaggcgtgtgatggttgaccctgagggtgaggttatgcgccaaaacgcgcgtaaattgaaggataagttggatcgaagcattgctcccggtggcagcagctacgagagcctggaacgcctgcagagctatattagcagcctg